European Patent Application EP 4 556 483 A1, published May 21, 2025. Title: Protein variant and method for producing L-lysine using the same. Applicant: CJ CheilJedang Corporation. The sequence listing filed with the application follows.

SEQUENCE LISTING (107 sequences)

SEQ ID NO: 1 - protein, 341 aa, synthetic construct
  REGION 1..341: note = protein variant of gene NCgl0030
MTKIKSGEASTSIVERALKRPELTSLLGAVLVFTLFMVVAPAFRSWDSMATVLYASSTIGIMAVAVGLLMIADEFDLSTGVAVTTAALAASMFSYNLWLNTWVGALIALVISLAIGFFNGFLVVKTKIASFLITLATFLMLQGINLAVTKLISGTVATPTIADMEGFPSARAVFASSIPIFGVIIRITVFWWLLFVIVGTFVLFKTRIGNWIFAVGGDEEAARAVGVPVRGVKIGLFMFVGFAAWFVGMHNLFLFDSIQAGQGVGNEFLYIIAAVIGGISMTGGRGTVVGTMIGALIFGMTNQGIVYAGWNPDWFMFFLGGTLLLAVLLNHRFERFNKERS

SEQ ID NO: 2 - protein, 536 aa, synthetic construct
  REGION 1..536: note = protein variant of gene NCgl0179
MHHEQPEGCEVGIRRTIPEESRTAFLDMINQGMSGLAASTAVGVSEFTGRKWAKAAGVKLTRGPRGGNAFDTAEKLEIAASMLEKGCLPREIGEYVGMTRANISLWRKQGPDKLRQRAATLRTGKRAAEFIHAPVMGPYYGPRTLHQVLREDYTTLFDELSALGLPAQVCGALLHLAPPPSLRFSYMSCVVPLFADEIKVVGQGTRLSLEEKMMIQRFHDTGVSAAEIGRRLGRCRQTISRELRRGQDDDGRYRARDSYEGAIRKLARPKTPKLDANRRLRAVVVEALNNKLSPEQISGLLATEHANDSSMQISHETIYQALYVQGKGALRDELKVEKFLRTGRKGRKPQSKLPSRGKPWVEGALISQRPAEVADRAVPGHWEGDLVIGGENQATALVTLVERTSRLTLIKRLGVNHGASTVTDALVEMMGDLPQALRRSLTWDQGVEMAEHARFSVVTKCPVFFCDPHSPWQRGSNENTNGLVRDFFPKGTNFAKVSDEEVQRAQDLLNYRPRKMHGFKSATQVYEKIVVGASTD

SEQ ID NO: 3 - protein, 260 aa, synthetic construct
  REGION 1..260: note = protein variant of gene NCgl0288
MGSITPQKRPRVGSHIANKGQETDIGRKRRARRINRTLTVAYPDAHCELDFTNPLELTVATILSAQCTDVRVNQVTPALFKRYPTVTDYANADRTELEEFIRPTGFYRNKATSLIGLGEALISLHDGQVPGTLEQLVELPGVGRKTANVVLGNAFGVPGITVDTHFGRLVRRLKLTDEEDPVKVEKVMNELIEKPEWTMFSHRLIFHGRRICHSRRAACGACMLAADCPSFGLEGPSDPFEAQKLIKSDDREHLLKMAGM

SEQ ID NO: 4 - protein, 478 aa, synthetic construct
  REGION 1..478: note = protein variant of gene NCgl0337
MELREYATILMKNWVLIVIASILGIAAGAGFSLLATPEYQSRTQLYVSVRSGAGTTSDMVQGANFSRQIVNSYVDVIKTGVVLEPVVDELGLELTANQLSSHISAASPADTALINITASSPSPQQAAEIANAVGESFKNVIQTELEPDSGDGMSPINLTTTQVALEPSSPVSPNVMMNILLGLLVGLAIGVGIAVLRAALDTRIHSLRDIEEVTDKPLLGGIIADSEVEKHPLIIKHKPHSPIAESFRALRTNLQFLNVGGSSSVFVISSANPGEGKSTTSVNLALALAEAGSRVALIEADLRLPRVSKYLGVEGNAGLTDILIGKAEVNDVLQRWGRTQLYYLPAGRIPPNPSELLGSAEMDKVIAELEESFDYVIIDAPPALAVTDAAVIGHGKAGILIAVSAGSTKKPELEATLSTLENADANVVGVVATMLPPKSVAGYGYGNYGYGDTSKINAPKPDNTELTTTDASKANNEQ

SEQ ID NO: 5 - protein, 318 aa, synthetic construct
  REGION 1..318: note = protein variant of gene NCgl0458
MSDENINEFEQDEDLNFGASFSDEFADDDFDAEADVEADAAAEASALEAEQDLEEETLDAPEEAAEEAPAAAESEAPVEEDEEADSLAQAAAALGDTDEQDADAEYKARLRKFTRELKKQPGVWYIIQCYSGYENKVKANLDMRAQTLEVEDDIFEVVVPIEQVTEIRDGKRKLVKRKLLPGYVLVRMDMNDRVWSVVRDTPGVTSFVGDEGNATPVKHRDVAKFLMPQEQAVVTGEAAAAAAEGEQVVAMPTDTKKPQVAVDFTVGEAVTILTGAFASVSATISSIDPELQKLEVLVSIFGRETPVDLSFDQVEKVS

SEQ ID NO: 6 - protein, 209 aa, synthetic construct
  REGION 1..209: note = protein variant of gene NCgl0627
MINHEVRTHRSAEEFPYEEHLAHKIARVAADPVEVAADTQEMIINRIIDNASVQAASVLRRPVSSARAMAQVRPVTDGRGASVFGLPGRYAAEWAALANGTAVRELDFHDTFLAAEYSHPGDNIPPILAAAQQAGKGGKDLIRGIATGYEIQVNLVRGMCLHEHKIDHVAHLGPSAAAGIGTLLDLDVDHHLPGNWSGIAHHHGDEAVP

SEQ ID NO: 7 - protein, 264 aa, synthetic construct
  REGION 1..264: note = protein variant of gene NCgl0686
MSTAYFIAHGNDTYRPTEHSSGAWRDDELHLAPVAGLVIHHMERWRREVVGDALVFSRFSLEVLGQIARDDVTLRTEIVRPGRTIELIETVAEINGRVTIRARAWLLKTSDLAHISGDTFEALPSMTELADVKSAFQWSGGFMDSIVFVEDAEKIPGKNRAWITGDVQLVDGEDSEPLAEFSKFLDVANGVAVREDPKTWMFPNVDLTFHLFRQPVGTKVGFDTRAAFGPNGIGLTTSVIHDAEGPVGTLNQSLTVRPIAELNK

SEQ ID NO: 8 - protein, 1532 aa, synthetic construct
  REGION 1..1532: note = protein variant of gene NCgl0706
MSAFDSILNVEEWISDHYLTNDDAKGASFSKRVRERIKEWKTTEDATQQSGPLTRFSSNRLQLQHALSELDDATTAASLVASALGYGVPSARHAQRGSDTISYSSWVGNAGSVEFLAATPAESFEENFRSLPLEPVAVNDKPQDITAAKLVGQIFLSDTPPAFVVITAGKWVVLAERETWPLGRHLAIDISLVVERNDTKAQGEMQQTVVALARENTERAADGTTWWEETIEQSREHAVKVSGELRSAVRESIEILGNDVLTRYEAKELSTAEIDGGELAKQSLRYLYRILFLLFAEASPELEILPTGTPEYDEGYGLARLRELILNPPVTQHARTGTHLYDSLQLLFTLVDKGHHPTDAKAVAFDAEAGEEGLHFRNLSADLFLPAATELIDRVGLSNEALNKVLENLLLSRVQSGKDRGFISYATLGVTELGQVYEGLMSYTGFIAQEDLFEVAPHGKADKGSWMLPVSKADEVPADSFIEVDQEAPGGGVIKVRKRHPRGSFVFRQSSRDRERSASFYTPQVLTSFTVTQAIEELQASKRITTANDVLSLTICEPAMGSGAFAVEAVRQLAELYLELRQEELEQQIPAEDRAKELQKVKAHIALHQVYGVDLNSTAVELAEISLWLDTMNAEMDAPWYGLHLRNGNSLVGATRSLYAPSLLNKKAWLTATPTRYRLDDIAQAIDENKAEPLFNHGIHHFLLPSTGWGATADAKDLKDLMATEIKELKSWRTSIRASLSKTQIKQLNNLALRVETLWRFVLMRIRIAESQISRSTTLWGQEPAEVSEVVTREQIEQDLFGNIDGAYNRLRLVMDAWCALWFWPLDAVATAEHPERPALPDLDEWLATLTEILGIDLPLKSKNENQIVLGPDTNWLAINDAEATDLGFSGALSFERVSANHPWINVARQVAKQQSFFHWDLDFAHVFAKGGFDLQVGNPPWVRPDVNFEDLLAEHDPWWAVMSKPTQASKKERQKNFHNNPKSLEHVVSGAGETVATSAILGSVTLYPHLKDQRPDLYRGFMEKTWSNASPAGAISLIHPESHFTEKKAAPLRRGAYERLRRHWQFINELILFDVHDLVKYGVHVYGAPQESINFLSAASLYHPQTVLDSFDHDGSGNLPGLKDDNGNWDRRPHKDRIQLVNADTLTVWKSILEDEQTPYLDTRMVYTVNTEAAAVLEKLASAPRIKELGLQFSSGWNETTDKKKGYFDVGWGYPASWSDAILQGPHLGVATPMIKQPNPTMKHNQDWSEIDFEAIPANFIPATAYQPDRQTKPTYDADYGTWTFGDKQVPVADTFRIAWREMAATTGFRTVYPSVIPPGANHVHTVNSAASRSNLKTILVGAQLGAILSDYFARSSGSSHIFNDIVRKIPLPNFTSLEKQFARTYLRLNCLTSAYAPLWEEITGEPWDVQVPLRNAEQRRAAQNDIDAMVALSLGISADELCMIYRTQFPVMRRYDQEDHFDANGRKVPKEIIKLQQKLKDGQELSVEKRTWVHPQSEVSYTFEYPFRVLDREADLRAAYAKFENQLKEP

SEQ ID NO: 9 - protein, 551 aa, synthetic construct
  REGION 1..551: note = protein variant of gene NCgl0799
MNSTILLAQDAVSEGVGNPILNISVFVVFIIVTMTVVLRVGKSTSESTDFYTGGASFSGTQNGLAIAGDYLSAASFLGIVGAISLNGYDGFLYSIGFFVARLVALLLVAEPLRNVGRFTMADVLSFRLRQKPVRVAAACGTLAVTLFYLIAQMAGAGSLVSVLLDIHEFKWQAVVVGIVGIVMIAYVLLGGMKGTTYVQMIKAVLLVGGVAIMTVLTFVKVSGGLTTLLNDAVEKHAASDYAATKGYDPTQILEPGLQYGATLTTQLDFISLALALCLGTAGLPHVLMRFYTVPTAKEARKSVTWAIVLIGAFYLMTLVLGYGAAALVGPDRVIAAPGAANAAAPLLAFELGGSIFMALISAVAFATVLAVVAGLAITASAAVGHDIYNAVIRNGQSTEAEQVRVSRITVVVIGLISIVLGILAMTQNVAFLVALAFAVAASANLPTILYSLYWKKFNTTGAVAAIYTGLISALLLIFLSPAVSGNDSAMVPGADWAIFPLKNPGLVSIPLAFIAGWIGTLVGKPDNMDDLAAEMEVRSLTGVGVEKAVDH

SEQ ID NO: 10 - protein, 483 aa, synthetic construct
  REGION 1..483: note = protein variant of gene NCgl1165
MTTALEEQNAQQAATAGRVVRVIGAVVDVEFPRGELPALYNALTVEVTLESVKKTVVLEVAQHLGDNLIRTIAMAPTDGLVRGAAVTDTARPISVPVGDVVKGHVFNALGDCLDDVSLNNNPEIERWGIHREPPSFDQLEGKTEILETGIKVIDLLTPYVKGGKIGLFGGAGVGKTVLIQEMITRIAREFSGTSVFAGVGERTREGTDLFLEMEEMGVLQDTALVFGQMDEPPGVRMRVALSGLTMAEYFRDVQNQDVLLFIDNIFRFTQAGSEVSTLLGRMPSAVGYQPTLADEMGVLQERITSTKGRSITSLQAVYVPADDYTDPAPATTFAHLDATTELDRSIASKGIYPAVNPLTSTSRILEPAIVGERHYEVSQRVIGILQKNKELQDIIAILGMDELSEEDKITVARARRIERFLGQNFFVAEKFTGLPGSYVPLTDTVDAFERICNGDFDHYPEQAFNGLGGLDDVEAAYKKLTGK

SEQ ID NO: 11 - protein, 481 aa, synthetic construct
  REGION 1..481: note = protein variant of gene NCgl1262
MTSPVENSTSTEKLTLAEKVWRDHVVSKGENGEPDLLYIDLQLLHEVTSPQAFDGLRMTGRKLRHPELHLATEDHNVPTEGIKTGSLLEINDKISRLQVSTLRDNCEEFGVRLHPMGDVRQGIVHTVGPQLGATQPGMTIVCGDSHTSTHGAFGSMAFGIGTSEVEHVMATQTLPLKPFKTMAIEVTGELQPGVSSKDLILAIIAKIGTGGGQGYVLEYRGEAIRKMSMDARMTMCNMSIEAGARAGMIAPDQTTFDYVEGREMAPKGADWDEAVAYWKTLPTDEGATFDKVVEIDGSALTPFITWGTNPGQGLPLGESVPSPEDFTNDNDKAAAEKALQYMDLVPGTPLRDIKIDTVFLGSCTNARIEDLQIAADILKGHKIADGMRMMVVPSSTWIKQEAEALGLDKIFTDAGAEWRTAGCSMCLGMNPDQLKPGERSASTSNRNFEGRQGPGDRTHLVSPAVAAATAIRGTLSSPADI

SEQ ID NO: 12 - protein, 929 aa, synthetic construct
  REGION 1..929: note = protein variant of gene NCgl1432
MSFSAEKGTHLSEFIADLGFDLDEFQIKGCHAVEEDHGVLVCAPTGAGKTIVGEFAVSLALSRGTKCFYTTPIKALSNQKYHDLVAKHGSDAVGLLTGDVSINHDADIVVMTTEVLRNMIYAGSFALERLSHVVMDEIHFLADASRGAVWEEVILNLDDSVNIIGLSATVSNSEEFGEWLTTVRGDTRVIVTDHRPVPLDQYMMVQRKVMPLFEPGTDGRVNKELEATIDRLNSKQSEQGRAAYRSGEGFRARSKGDKQDSRTGKPREQDRHRPLGRPEVLSILKGINMLPAITFIFSRAGCDGALYQCLRSKLVLTDQAESEEIARIVDAGVVGIPEEDLQVLNFKQWRAALMRGFAAHHAGMLPAFRHIVEELFVKGLVRAVFATETLALGINMPARTVVLEKMVKFDGEGHVDLTPGQYTQLTGRAGRRGIDVLGNAVVQWSPALDPRWVAGLASTRTYPLISTFQPGYNMSVNLLKTIGYEPSLRLLEKSFAQFQADGSVVGDVREIERAEAKVAELRAQLNKEIAATNPAVREDQDAVEVFIDYMELRRELNEEEKLNRKQSIEDRNVETVRVLSKLQIGDVIAMPGRKRPVLAVVMTPANQSRDPRPWVTTESGWSGRVDAESFTNPPITIGHMRLPRQAIEEPRRNARRVQELFRREHFKRPNKMREFARVRPNEAVTKLRNAIRDHEAYHWPDREHLARTAERMIRKERDLAKLTGNVDKARETLGRTFERILSLLSEMDYVDYSNPDNPVITDEGERLAKIHSEADLLVAQCLKRGIWDNLDPAELAGVVSMCTFENRRETGGEAQAVTEAMADSMNSVERIWGELVEDERRHRLPITRQPEAGFATAIHQWASGAPLGYCMAAAAENGAELTPGDFVRWCRQVIDLLEQVAKTAYFDETTRNARQAIDAIRRGVVAIGS

SEQ ID NO: 13 - protein, 193 aa, synthetic construct
  REGION 1..193: note = protein variant of gene NCgl1531
MTTNAPDGATNNINNAHSGAVGKPKVQLSDAEIQKYTAAFAGTTTTKPWELEVTTKFLKKIAWVAVVVIMAVHIFMGAVVDVDFTGAAVTFVDTLAFPALGIIFSVLVFLGLTRPRVRANEDGVEVRNFIGTRFYPWVVIYGMSFPKGSSVARLELPDFEFVPMWAFQSRDGEDVVRAVATFRDLENKYMPED

SEQ ID NO: 14 - protein, 185 aa, synthetic construct
  REGION 1..185: note = protein variant of gene NCgl1588
MKLFSRTSLVALGTAAAITLSGVTAPAFADEDSNAAVSALKTAEDNTPEAPGASTPLKLEQPGTITGVPGKAITPVTVKVIAGEAESFTSDNLPSGLLIDNTGKITGTPKKEFTGSAKIIAKNEAGVEAEVYVNFDFNEEPSSEEPSSGSSDTDNIENWIKIITAVIGALTTILTFSTKLDSFLK

SEQ ID NO: 15 - protein, 264 aa, synthetic construct
  REGION 1..264: note = protein variant of gene NCgl1859
MVSQTERQHAIASLLAPTGAVSVGDLAEHFHVTTETVRRDLRIMESLGLLQRVHGGAISPEPMGTSPPRLKPALVKGMPPEPRVLELAETAVSLITPLARSIFLDSGLACTAIATVLGDPPEDARWTVVTSSPGAVIALSATDATSTVVLHGQVHGNCSSIIGSTAVDMISQLRADIAFVEVDAIQSDTSLCTFFPETIPIKQAMIKNAAFTVAVLSPRSPQDQELQLLKHPFSTLADFDALVTDDHTLDFPVLPDHNFQVVTP

SEQ ID NO: 16 - protein, 526 aa, synthetic construct
  REGION 1..526: note = protein variant of gene NCgl1874
MTQQLNHAKVNQHPGQATLPETAEGQVRTYEVKTYGCQMNVHDSERLSGLLEEAGYVAAPEDTTPDLVVFNTCAVRENADMRLYGTLGNLRSVKEKNPGMQIAVGGCLAQKDKDTVVKKAPWVDVVFGTHNIGSLPTLLQRAEHNAQAEVEIVDSLEQFPSVLPAKRESAYAGWVSVSVGCNNTCTFCIVPSLRGKEQDRRPGDILAEVQALVDQGVTEVTLLGQNVNAYGVNFVDPELERDRSAFSKLLRACGEIEGLERVRFTSPHPAEFTSDVIDAMAETPNICPQLHMPLQSGSDKVLKEMRRSYRSKKFLSILDEVRAKIPHASITTDIIVGFPGETEEDFQATLDVVKKARFTSAYTFQYSPRPGTPAAEYENQLPKEVVQERYERLMVVQEQVCEEENQKLIGTTVELLVQAGGGRKNDATKRMSGRARDGRLVHFAPEGDIDGEIRPGDFVTVTVTEAKPFFLIADSGVQTHRRTKAGDNSAVGQVPTTAPIGVGLGLPQIGAPKVAPATESACCSIN

SEQ ID NO: 17 - protein, 38 aa, synthetic construct
  REGION 1..38: note = protein variant of gene NCgl3069
MAVAKDVLSFSRPIPALHAIIGALGWFGMFAVSLWSTL

SEQ ID NO: 18 - protein, 517 aa, synthetic construct
  REGION 1..517: note = protein variant of gene NCgl2356
MSITTHVQALTTALNAIDNHLASMLDHGVTPDQYKAIEPDLIALEHTINHHATIAAQTTALAERTNAAHTIGSTHLIDYLTTTFGLSKARAHHRINLAHSLYPIPKPNPGSGNGGNGGNPDGGPDGGDSGDDDSGDDDPDPEPDKPEDGKPDGDKPRGPRISAEKHAIITDELARLNPNTTPSAEELRTQALSQAIWRTPEDLRTWLRHHVTTANKNNPNPITAMKRRYLAVGKPDADNMVRISGLVPAATAALITANTAPLTKRGNLVDLPAAEDMRTRGQRHADALHHIMEIYNHGIVTPARGGTASIIISMTTDDLDEINHGDHGDGSLLNNLYPTNTGYSLNLAEIMNLIAAKYDFAVLLDGETGQPLNVNRMQRSANLTQRIALFASELVCSAPNCDRPQLECEVHHLDPWMRGGLTNLVNLTHQCFNHHPRNDDSRSGVNGKGFMDRDPATGRVGHYPVGGEGPVFNRSAAADRSGGAWARRKHHGPPPTPPDPPDPPGPEPDPGDEGRLF

SEQ ID NO: 19 - protein, 41 aa, synthetic construct
  REGION 1..41: note = protein variant of gene NCgl3082
MRMLFENSIVCHLLFLSLPQITLGDVWWVMPGGGSPNYRSL

SEQ ID NO: 20 - protein, 481 aa, synthetic construct
  REGION 1..481: note = protein variant of gene NCgl2542
MPKPLPPETRRKIIDFDPFAPNSPSIEEFCSRLKISRRSFYNIRNRYQQDANAALHPHSSAPITARRTYDESITSTLLSIRARLKAQGWEYGPISIRFEGISTGELTAPIPSVSTIARLLRAAGAVESNPKKRPKSSVVRFQRGQAMEMWQIDGFIYTLHDTDLTRVTIYQILDDATRFDVGTCVFPANENSVDARTALEQAIAHFGAPHELLSDNGSAFNRMRQGYVGSLESYLATVGCLSITGKPGHPQTQGKNERSHRTLFRFLQAHQPHTLEECAHYIEQFRDHYNNRRPHQGLPNNLSPAAAWEIVGCVEQQPPIDPVVLQQQADHYARRRIEKQSDVPLVRQEESVPVSKMQQTEQRRRVRRFGKKPVDPDVFTFAGNNQKVVFQGMRISVPRTMRDREFYRTVTATELGFWDAITGELELSIPLPVVAIARGKSYINSYNIRGVWMQHPTPLWQRKRDEAEKRFKSIDPGDLLR

SEQ ID NO: 21 - protein, 610 aa, synthetic construct
  REGION 1..610: note = protein variant of gene NCgl2765
MTTAAIRGLQGEAPTKNKELLNWIADAVELFQPEAVVFVDGSQAEWDRMAEDLVEAGTLIKLNEEKRPNSYLARSNPSDVARVESRTFICSEKEEDAGPTNNWAPPQAMKDEMSKHYAGSMKGRTMYVVPFCMGPISDPDPKLGVQLTDSEYVVMSMRIMTRMGIEALDKIGANGSFVRCLHSVGAPLEPGQEDVAWPCNDTKYITQFPETKEIWSYGSGYGGNAILAKKCYALRIASVMAREEGWMAEHMLILKLINPEGKAYHIAAAFPSACGKTNLAMITPTIPGWTAQVVGDDIAWLKLREDGLYAVNPENGFFGVAPGTNYASNPIAMKTMEPGNTLFTNVALTDDGDIWWEGMDGDAPAHLIDWMGNDWTSESDENAAHPNSRYCVAIDQSPAAAPEFNDWEGVKIDAILFGGRRADTVPLVTQTYDWEHGTMVGALLASGQTAASAEAKVGTLRHDPMAMLPFIGYNAGEYLQNWIDMGNKGGDKMPSIFLVNWFRRGEDGRFLWPGFGDNSRVLKWVIDRIEGHVGADETVVGHTAKAEDLDLDGLDTPIEDVKEALTAPAEQWANDVEDNAEYLTFLGPRVPAEVHSQFDALKARISAAHA

SEQ ID NO: 22 - protein, 433 aa, synthetic construct
  REGION 1..433: note = protein variant of gene NCgl2816
MTTAVDQNSPPKQQLNKRVLLGSLSGSVIEWFDFLVYGTVAALVFNKMYFPSGNEFLSTILAYASFSLTFFFRPIGGVIFAHIGDRIGRKKTLFITLMLMGGGTVAIGLLPDYNAIGIWAPILLMFLRILQGIGIGGEWGGALLLAYEYAPKKQRGLYGAVPQMGISLGMLLAAGVISLLTLMPEDQFLTWGWRIPFVGSILLVFIGLFIRNGLDETPECKRIRDSGQQVKMPLKEVLTKYWPAVLVSIGAKAAETGPFYIFGTYIVAYATNFLNIRDNIVLLAVACAALVATIWMPLFGSFSDRVNRAVLYRICASATIVLIVPYYLVLNTGEIWALFITTVIGFGILWGSVNAILGTVIAENFAPEVRYTGATLGYQVGAALFGGTAPIIAAWLFEISGGQWWPIAVYVAACCLLSVIASFFIQRVAHQEN

SEQ ID NO: 23 - DNA, 1026 bp, synthetic construct
  misc_feature 1..1026: note = nucleotide variant of gene NCgl0030
  source 1..1026: mol_type = other DNA
atgacaaaaatcaagagtggggaggcgtcgacaagcattgttgagcgcgccttaaagcgccccgaactgaccagcctgcttggcgccgtgcttgtttttacgctgtttatggtggtcgcgccggcatttaggtcatgggattcgatggcgaccgtgctgtatgcgagttccacgatcggcatcatggcggttgccgtgggcctgctgatgatcgctgatgaattcgacctgtccaccggcgttgccgtgacaactgcagcgctggcggcctcgatgtttagctataacctgtggctgaacacctgggtgggcgcgctgattgcattggtgatttcgctggccatcggctttttcaacggctttttggtagtgaaaaccaagattgcatccttcctgatcacccttgccactttccttatgctgcagggtattaatctggcggtcaccaagctgatttccggcaccgtggccacgccaaccatcgcggatatggaaggttttccttcagcgcgtgcggtgtttgccagctcgattcccatctttggtgtgattattcgcatcactgttttttggtggctgctgtttgttatcgtcggcacttttgtgttgtttaagacgcgcatcggcaactggatttttgcggtcggtggcgatgaagaggcagctcgcgcagtcggcgttcccgtgcgtggcgtgaaaatcggcctgttcatgttcgttggttttgccgcctggtttgtgggcatgcacaacctgttcctctttgattcgattcaggctggtcaaggcgtgggtaatgagttcctctacatcatcgctgcggtgatcggaggcatctccatgactggtggccgcggaacagtggtgggcacaatgattggtgcactcatctttggaatgaccaaccaaggcattgtttatgcaggttggaaccctgactggttcatgttcttcctcggcggcaccctacttctggctgttttgctcaatcaccgattcgagcgtttcaacaaggagcgatcatga

SEQ ID NO: 24 - DNA, 1611 bp, synthetic construct
  misc_feature 1..1611: note = nucleotide variant of gene NCgl0179
  source 1..1611: mol_type = other DNA
atgcaccacgagcaacccgaagggtgcgaagtgggcattcgtagaacaatcccagaggaaagccgtacggctttcctcgacatgatcaatcaaggtatgtcaggtcttgctgcgtctacagcggtcggggtcagtgaattcaccgggcgaaagtgggcgaaggccgccggggtgaaactgacccgcggcccgcgaggtggcaatgcttttgacaccgccgagaaacttgagattgcagccagcatgctagagaaaggatgcctaccccgagaaatcggcgagtatgtcggcatgactcgggccaatatatccctatggcgcaaacaaggcccagacaagcttcgccaacgcgcagccaccttgcgcaccggcaagcgagcagctgaattcatccacgccccggtgatgggcccttattatgggccacgcacactccatcaagtgttgcgtgaggactacacaacactgtttgacgagttatctgcgttggggttgccagcacaggtgtgtggggccttacttcatcttgctccaccaccatcattacgcttttcttatatgtcgtgtgtagtgccgttatttgctgatgaaatcaaagtcgtaggacaaggcacacgattatcgttagaagagaaaatgatgatccaacgtttccatgacaccggggtcagtgcagcagaaatcggtcgacgcctgggtcggtgtcggcaaacaatttccagggaacttcgacgtggtcaagatgatgatggacgttatcgtgcacgcgactcctatgaaggtgcgatcaggaaactagcgcgtccgaaaacaccgaaacttgatgccaatcgtaggcttcgggctgtggtggtcgaggcgttgaataataaattatctccggagcagatttctggtcttttagccaccgagcatgctaacgatagctctatgcagattagtcatgaaactatttaccaggcgttatatgttcaaggtaaaggggcgttgcgtgatgaattgaaggtggagaaatttcttcgtaccggtcggaagggacgtaaaccgcagtcgaagttgccatcgagaggtaagccgtgggtggagggtgcgttgattagtcaacgcccagcagaagttgctgatcgtgctgtgcctgggcactgggagggcgatttagtaattggtggtgaaaaccaagcgacagcgttggtgacgttggtggagcgcacgagccggttgacgttgattaagcggttgggggttaatcatggggcgtcgactgtgacggatgcgttggtggagatgatgggtgatttgccgcaggcgttgcgtcggagtttgacgtgggatcagggtgtggagatggcagagcatgcgcggtttagcgtggtgaccaagtgtccggtgtttttctgtgatcctcattcgccgtggcagcgtgggtcgaatgagaatacgaatggattggtcagggattttttcccgaagggcactaattttgctaaagtaagtgacgaagaagttcagcgggcacaggatctgctgaattaccggccgcggaaaatgcatggttttaaaagcgcgacgcaggtatatgaaaaaatcgtagttggtgcatccaccgattga

SEQ ID NO: 25 - DNA, 783 bp, synthetic construct
  misc_feature 1..783: note = nucleotide variant of gene NCgl0288
  source 1..783: mol_type = other DNA
atgggttccattactccgcagaagcggcctcgcgtggggtctcacatcgcgaacaagggtcaagagactgatatcgggcgaaaacgccgagctcgacgcatcaatcgcacactcaccgtggcatatccggatgcgcactgcgaattagatttcaccaatccgctagaactcacggtcgccaccattttgtccgcccagtgcacggacgttcgcgtgaaccaggtgacgcccgcgttgttcaagcgctatccgacggtcacagattacgccaacgccgatcgcacggaattggaggagttcatccgtccgacaggcttttaccgcaacaaggccacttctttaatcggcctgggtgaggcactaatttcgcttcacgacggccaggtccccggtacccttgagcagctagttgagctgccgggggtcgggcggaaaaccgccaacgtggtgctgggaaatgctttcggtgttccgggaatcacggtggatacacactttggcaggttggtgcgtcgcctgaagctcactgatgaagaagatcccgtcaaggtggaaaaagtgatgaacgaactcatcgaaaagcctgagtggaccatgttttcacataggctgatcttccacggacgtaggatatgtcatagtcgacgcgccgcctgtggagcctgcatgctggcagctgattgcccatcctttggtttggaggggccgtcagatccatttgaggcgcaaaaactcattaaaagtgatgatagggagcacctgctgaaaatggcaggaatgtag

SEQ ID NO: 26 - DNA, 1437 bp, synthetic construct
  misc_feature 1..1437: note = nucleotide variant of gene NCgl0337
  source 1..1437: mol_type = other DNA
atggaattaagggaatacgcgacaatcctgatgaagaattgggtgttgatcgttatcgcatccattcttggaattgcagcgggcgctggtttttcccttctagctacaccggagtatcagtcacgtactcagttgtatgtatcggtgcggtcgggggctgggacaacctctgacatggttcagggtgctaacttttcgcgtcagattgtgaatagttatgttgatgtcattaagacgggtgttgttctagagccggttgttgatgagcttggtctggagttgacggctaaccagttgagttctcatatcagtgcggcttctcctgctgatactgcgttgatcaacatcactgcttctagtccttctcctcagcaggcggctgagatcgccaatgcagtgggggagagtttcaagaatgtgattcagactgaattggaaccagactccggcgatggcatgagcccgattaacctgactactactcaggtggctctggaaccatcttctccggtcagtcctaatgtgatgatgaatatcctcctcggcctacttgtaggtcttgcaataggtgttggtattgcagtgcttcgcgcggctttggatactcgtattcattccttgcgcgatattgaagaggttactgataagccacttttgggcggaatcattgcggattctgaagttgagaagcacccgttgatcattaagcacaagccgcatagtcctattgcggagtcctttcgtgcgttacgtactaacctgcagttccttaacgtcggcggctcatcttcagtatttgttatctcctctgctaatcctggtgagggtaagtcaaccacttctgtaaacctagctttggcgcttgcagaggccggctcccgtgtagcgctgatcgaagctgatcttcgcttgccacgagtgagcaagtacctcggagttgagggcaacgcaggtctgactgacattctcattggcaaggccgaggttaatgatgtgttgcagcgttggggtaggactcagttgtactatctcccggcagggcgcattccgccgaacccgagtgagttgcttggttcagctgagatggacaaggtcattgcggagcttgaggaaagctttgattatgtgatcatcgatgcccctccggcgttggcggttaccgatgctgcagttattggtcatggcaaggctggcatcctgattgcggtctccgcaggttctacaaagaagcctgagttggaagctacgctgtccacgcttgagaatgcggatgccaatgttgttggcgttgtcgctacgatgctcccgcctaagtctgtggctggttatggctacggaaattacggctacggcgacacctccaaaatcaatgcccctaagcccgacaacaccgaactaaccaccaccgatgcttccaaggccaacaatgagcaatag

SEQ ID NO: 27 - DNA, 957 bp, synthetic construct
  misc_feature 1..957: note = nucleotide variant of gene NCgl0458
  source 1..957: mol_type = other DNA
atgagcgatgagaacattaacgagtttgagcaggacgaggatctgaacttcggcgcgagctttagtgatgaattcgcagatgacgatttcgatgcagaagcagacgtagaagcagatgctgctgcagaggcctctgccctggaagctgagcaggatctggaagaagagaccctagatgctccagaagaagccgcagaagaagctcctgctgctgcagagtccgaagctccagtagaagaggacgaagaggctgacagccttgctcaggcggctgctgcacttggtgacaccgatgagcaggacgcggatgcagagtacaaggctcgtctgcgtaagttcactcgtgagctgaagaagcagcctggtgtttggtacatcattcagtgctactccggctacgagaacaaggtgaaggcgaaccttgacatgcgtgctcagacccttgaggttgaggatgacatctttgaggttgttgttcctatcgagcaggtcactgagatccgtgatggtaagcgcaagctggttaagcgtaagttgctgccgggctacgttttggtccgcatggacatgaatgaccgcgtgtggtctgttgttcgcgatacacctggtgtgaccagctttgtgggtgacgagggcaatgcaactcctgtgaagcaccgcgatgttgcgaagttcttgatgcctcaggagcaggctgttgtcaccggtgaggctgctgctgcggctgccgagggtgagcaggttgtggctatgcctaccgataccaagaagcctcaggttgctgtggacttcactgttggtgaggctgtgaccattctgactggtgctttcgcttctgtttctgcaacgatttcttctatcgatcctgagctgcagaagctggaagttttggtgtccatctttggtcgtgaaactcctgttgatctcagcttcgaccaggttgagaaggttagctag

SEQ ID NO: 28 - DNA, 630 bp, synthetic construct
  misc_feature 1..630: note = nucleotide variant of gene NCgl0627
  source 1..630: mol_type = other DNA
atgattaaccacgaagtgcgcacccaccgttctgcggaagagttcccgtacgaggagcacctggctcacaagatcgctcgcgttgcagccgacccagttgaggttgctgcggacactcaggaaatgatcatcaaccgcatcatcgacaatgcatcggtgcaggcagcttccgtgttgcgtcgaccagttagctctgcccgtgcgatggcacaggtcaggccagttaccgatggtcggggtgcatctgttttcggtctgccaggacgttatgccgcggaatgggctgcgcttgctaacggcactgcggtgcgtgagcttgatttccatgacacgttcctcgctgcggaatactcccacccaggagataacattcctccgattttggctgcagcacagcaggctggaaaaggtggcaaggatctgatccgtggcatcgctactgggtatgagattcaggttaacttggtgcgtggaatgtgcctgcatgagcacaagattgatcacgttgctcatcttggaccatcagcggctgctggtatcggaaccttgctagacctagatgtggaccaccatctaccaggcaattggtcaggcattgcacaccaccacggcgacgaggcagtcccgtaa

SEQ ID NO: 29 - DNA, 795 bp, synthetic construct
  misc_feature 1..795: note = nucleotide variant of gene NCgl0686
  source 1..795: mol_type = other DNA
atgtcaactgcatattttattgcgcacggaaacgatacgtaccgcccaacggagcattccagcggtgcgtggcgcgatgatgaactccaccttgcaccggttgccggtttggtgattcaccatatggaacgttggcgcagggaagtggttggcgatgctttggtgttcagccgttttagtttggaggtcttgggccagatcgctcgggatgatgtcaccttgagaacagagatcgttcgtcccgggcgcaccattgaacttattgaaaccgtggctgaaatcaacggcagagtgacgattcgtgcacgcgcctggttgctgaagacctctgatcttgcccatatttctggcgatacttttgaagcgttgccgtcaatgactgaactggcagatgttaagtcagcgttccagtggtctggtggatttatggacagcattgtgtttgttgaggacgctgagaaaattccgggcaaaaaccgcgcgtggattaccggcgatgtgcagttggttgacggcgaagattctgagcctttggcagagttttccaaattcttggatgtggccaatggcgtggcggttcgggaagatccaaagacttggatgttcccgaacgtggatcttactttccatctgttccgccagccggtgggcaccaaggtgggttttgatacccgcgcggcgtttggacccaacggcatcggtttgaccacgtcggtgattcacgatgccgaaggtcctgtgggcacgcttaatcaatcattgacagtgcgcccaattgctgagttaaacaagtga

SEQ ID NO: 30 - DNA, 4599 bp, synthetic construct
  misc_feature 1..4599: note = nucleotide variant of gene NCgl0706
  source 1..4599: mol_type = other DNA
atgagtgcatttgattcgatcctaaatgttgaagagtggatcagtgaccactacctcaccaatgacgatgccaaaggtgcctcattttccaagcgggtgcgcgagcgcattaaagaatggaaaaccaccgaggacgcaacccagcagagtggccctttaactcgtttttccagcaaccgcctgcagttgcagcatgctctttctgagcttgacgacgccaccaccgccgccagtttagtggcctctgcactggggtatggtgtccccagcgcgcgccacgcgcagcgcggctccgacacaatatcctattcctcttgggtgggaaatgccggcagtgtggaatttcttgcagcgactcccgctgaaagctttgaagagaacttccgatcccttccccttgagccagtagcggtcaatgacaagccccaggatatcaccgcagccaaattggtgggccagattttccttagtgatactccccctgcttttgttgttatcaccgctggtaaatgggtggttttagccgagcgtgaaacctggcctctaggccgccacctagctattgatatttccctggtggtggaacgtaatgacaccaaagcccagggtgagatgcagcagacggtcgtagcactagcccgcgaaaataccgagcgtgccgccgatggcaccacctggtgggaagaaaccattgagcaatcccgcgaacatgctgtcaaggtttctggcgagctacgcagtgcggtgcgtgaatccattgaaatcctgggcaatgacgtgctcacacgctatgaagctaaagagctctccaccgctgagatcgacggtggcgagctagctaagcaatctttgcgctatctctaccgcattttgttcctgctttttgccgaggcttcaccagagcttgaaatcctgccaaccggcaccccggaatatgacgagggttatggcttggcacgcctgcgcgagcttattcttaatcccccagttacccagcatgctcgcacgggcacccacctttatgattccctgcagctgctgttcactctggtggataaaggccaccacccaacagatgctaaggctgtagcttttgatgccgaggctggagaagaaggcctgcacttccgcaacctttcagcggatctcttcctccctgcagccacagaacttattgatcgagttggtctttccaatgaagccctaaacaaggtcttggaaaacctcctgctctcccgggtgcaatccggtaaagaccgcggctttatctcctatgccaccttgggtgttaccgagcttggccaagtttatgagggtctgatgtcctataccggctttatcgcccaggaagatctttttgaggttgcaccacatggcaaagccgataaaggttcctggatgctcccggtctcaaaggctgatgaagtccctgccgatagctttatcgaagttgatcaagaagcccctggtggcggcgtaatcaaggtgcgtaaacgccacccgcgcggatcatttgtgttccgtcagtcctctcgtgaccgcgaacgctcagcgtccttctacaccccacaagtactcaccagctttactgtcacccaggctattgaagaactccaggcatcaaagcgcatcaccacagccaatgatgttctcagcctcaccatctgtgaacctgccatgggttccggcgccttcgctgtggaagcagtacgccaattagcagagctttatttggaattgcgccaagaagaactagagcagcagattccagcggaagaccgtgccaaggaactccaaaaggtcaaagcgcacattgcgctgcaccaggtttatggtgtggaccttaacagcactgctgtggagttggcggaaatctcgctgtggctagacaccatgaatgcagaaatggacgcaccttggtatggcctgcacctgcgtaatggtaactccctcgttggtgccacccgttcgctgtatgcacctagtctgcttaataaaaaagcctggttaactgctactccaacccgctatcggcttgatgatatcgcgcaggctattgatgaaaacaaagcagaacccctcttcaaccacggcatccaccacttcctcttgccctctactggctggggagccactgcagatgccaaagatcttaaagatcttatggctactgaaatcaaggagcttaaatcttggcgtacttccatccgtgcgtctttgagtaaaactcagattaagcagctcaataaccttgccctacgcgtggaaacactatggcgatttgtgctgatgcgtattcgcattgcagaatcccagatctcacgtagcactactctctggggtcaagagccagctgaggtttcggaggttgtcacacgtgagcaaattgaacaagacctctttggcaatattgatggtgcatataaccgtctacgcttggtgatggatgcttggtgtgcgctgtggttctggcctttggatgctgttgctaccgctgagcatccggagcgtccagcccttccagatcttgatgagtggctagccaccctgacggagattctgggtattgatctccctctgaagtccaaaaacgaaaatcagattgtcttaggtccagataccaattggctagccattaatgatgccgaggctactgatcttggtttttctggggcattgagctttgagcgtgttagcgcgaatcacccgtggatcaatgttgcccgccaagtggctaaacaacagagcttcttccactgggatctagacttcgcccacgtttttgccaagggtggatttgatctgcaggttggtaatccaccatgggtgcgaccagatgtgaactttgaggatctgcttgctgaacatgatccgtggtgggctgtaatgagtaaaccaacccaggcatccaaaaaagaacgccagaagaattttcacaacaatcctaagagcctcgaacatgtggtcagtggtgcaggtgaaaccgtggctacttctgcgatcctcggttcggttactctctatccgcatcttaaagatcaacgcccggacctctaccggggctttatggaaaagacttggtctaatgcctccccggcaggtgcgatctcactgatccaccccgaatcccacttcactgagaaaaaagctgccccgctacgtcggggagcatatgagcgtctgcgccgccactggcagttcattaatgagttgattctttttgacgtccacgacttggttaaatatggcgtacatgtctatggcgctccgcaggaatctattaactttttaagtgctgcgtcgctttatcacccacaaacagtgcttgattcatttgatcatgacggttcaggtaatctccctggtcttaaagacgacaatggcaactgggaccgtcgcccacacaaggaccgtatccaactggtcaatgccgatactttgacggtgtggaagtccatcctggaggatgaacaaacgccatacttggatacccgcatggtttataccgtcaacacggaagcagcagcagtgttggaaaagttggcttctgcacctcgtatcaaagaactcgggctgcagttctccagtggctggaatgaaaccaccgataagaaaaagggatactttgacgttggttggggctacccagcttcctggtctgatgccattttgcaggggccgcacctgggtgttgctacaccaatgatcaagcagcccaatccgacaatgaagcataatcaagattggtctgaaattgatttcgaggccattcctgcaaacttcatacctgcaacggcgtaccagcccgatcgccaaacaaagcccacttatgatgctgactacggcacctggactttcggggacaagcaggtaccagttgcagacactttccgaattgcatggagggagatggctgccaccacgggatttaggactgtctacccatcagtaattccaccgggagccaaccatgtgcacacagttaatagcgctgcatcacgttcaaacttaaaaaccattctcgttggagcacagcttggtgcaattctaagtgactattttgctcggtcctcgggttcaagccacatatttaacgacattgttcgcaagattccacttccaaatttcacatccttggaaaagcagttcgcccgcacatacctccgcctcaactgcctgacctcagcttatgccccattgtgggaagagatcaccggtgagccgtgggatgttcaggtgcctttgcgcaatgccgagcaacgtcgagcagcgcaaaacgatattgatgccatggtggcattgtctttgggtattagtgctgatgagctgtgcatgatttatcgcactcaattcccagtgatgcgtagatatgatcaagaagatcattttgatgccaatggccgtaaagttcctaaagagatcatcaagctgcagcagaaacttaaagatggccaagagctcagcgtggaaaagcgcacctgggtgcatccccaatcagaagtgtcctatacctttgaatatcctttccgggtgttggatcgtgaagctgatctgcgtgctgcatatgcaaaatttgaaaaccagctaaaggagccatag

SEQ ID NO: 31 - DNA, 1656 bp, synthetic construct
  misc_feature 1..1656: note = nucleotide variant of gene NCgl0799
  source 1..1656: mol_type = other DNA
atgaattccactattctccttgcacaagacgctgtttctgagggcgtcggtaatccgattcttaacatcagtgtcttcgtcgtcttcattattgtgacgatgaccgtggtgcttcgcgtgggcaagagcaccagcgaatccaccgacttctacaccggtggtgcttccttctccggaacccagaacggtctggctatcgcaggtgactacctgtctgcagcgtccttcctcggaatcgttggtgcaatttcactcaacggttacgacggattcctttactccatcggcttcttcgtcgcaaggcttgttgcactgctgctcgtggcagagccacttcgtaacgtgggccgcttcaccatggctgacgtgctgtccttccgactgcgtcagaaaccagtccgcgtcgctgcggcctgcggtaccctcgcggttaccctcttttacttgatcgctcagatggctggtgcaggttcgcttgtgtccgttctgctggacatccacgagttcaagtggcaggcagttgttgtcggtatcgttggcattgtcatgatcgcctacgttcttcttggcggtatgaagggcaccacatacgttcagatgattaaggcagttctgctggtcggtggcgttgccattatgaccgttctgaccttcgtcaaggtgtctggtggcctgaccacccttttaaatgacgctgttgagaagcacgccgcttcagattacgctgccaccaaggggtacgatccaacccagatcctggagcctggtctgcagtacggtgcaactctgaccactcagctggacttcatttccttggctctcgctctgtgtcttggaaccgctggtctgccacacgttctgatgcgcttctacaccgttcctaccgccaaggaagcacgtaagtctgtgacctgggctatcgtcctcattggtgcgttctacctgatgaccctggtccttggttacggcgctgcggcactggtcggtccagaccgcgtcattgccgcaccaggtgctgctaatgctgctgctcctctgctggccttcgagcttggtggttccatcttcatggcgctgatttccgcagttgcgttcgctaccgttctcgccgtggtcgcaggtcttgcaattaccgcatccgctgctgttggtcacgacatctacaacgctgttatccgcaacggtcagtccaccgaagcggagcaggtccgagtatcccgcatcaccgttgtcgtcattggcctgatttccattgtcctgggaattcttgcaatgacccagaacgttgcgttcctcgtggccctggccttcgcagttgcagcatccgctaacctgccaaccatcctgtactccctgtactggaagaagttcaacaccaccggcgctgtggccgctatctacaccggtctcatctccgcgctgctgctgatcttcctgtccccagcagtctccggtaatgacagcgcaatggttccaggtgcagactgggcaatcttcccactgaagaacccaggcctcgtctccatcccactggcattcatcgctggttggatcggcactttggttggcaagccagacaacatggatgatcttgctgccgaaatggaagttcgttccctcaccggtgtcggtgttgaaaaggctgttgatcactaa

SEQ ID NO: 32 - DNA, 1452 bp, synthetic construct
  misc_feature 1..1452: note = nucleotide variant of gene NCgl1165
  source 1..1452: mol_type = other DNA
atgactacagctcttgaagagcagaacgcacagcaggcagccactgccggccgtgtcgtgcgtgtcattggtgcggtcgtcgacgtggagtttccccgcggcgagctgccagcactgtacaacgcacttactgtagaggtaaccctcgaatcagttaagaagaccgttgttctcgaggttgctcagcacctcggcgacaacctcatccgcaccatcgctatggcaccaaccgacggacttgtccgcggtgctgctgtaaccgatactgcacgcccaatttccgtaccagtgggcgatgttgttaagggccacgtattcaacgctttgggcgactgcctagacgacgtttccctgaacaacaacccagagatcgagcgttggggcatccaccgcgagccaccatcattcgatcagcttgagggtaagaccgagatcctggaaacaggcatcaaggttatcgaccttctcaccccttacgttaagggtggaaagatcggcctcttcggtggtgcaggtgtgggtaagaccgttcttatccaggaaatgatcacccgtattgcacgtgagttctccggtacttccgtgttcgcaggtgttggtgagcgtacccgtgagggcaccgacctcttcctcgaaatggaagaaatgggcgttctccaggacaccgccctggtgttcggtcagatggatgagccaccaggagtccgtatgcgcgtggctctgtccggcctgaccatggcggagtacttccgcgatgttcagaaccaggacgtgctgctgttcatcgacaacatcttccgtttcacccaggcaggttctgaggtttccacccttctgggtcgtatgccttccgccgtgggttaccagccaaccctggctgacgagatgggtgttctccaggagcgcattacctccaccaagggccgttcgattacctctctgcaggccgtttacgttcctgccgatgactacaccgacccggctccagcgaccaccttcgctcacttggatgcaaccaccgagcttgaccgctccattgcttccaagggtatttacccagcagtgaacccactgacctccacctctcgtattctcgagccagcaatcgttggtgagcgtcactacgaggtttctcagcgtgtcatcggcattctgcagaagaacaaggaacttcaggacatcatcgccatccttggtatggacgagctttctgaagaggacaagatcaccgttgcacgtgcgcgtcgcatcgagcgcttcctgggtcagaacttcttcgttgcagagaagttcaccggtcttcctggctcctacgtgccactgaccgacaccgtcgacgctttcgagcgtatttgcaacggcgacttcgaccactacccagagcaggctttcaacggcctcggtggtttggacgatgtcgaagctgcatacaagaagctgaccggaaagtaa

SEQ ID NO: 33 - DNA, 1446 bp, synthetic construct
  misc_feature 1..1446: note = nucleotide variant of gene NCgl1262
  source 1..1446: mol_type = other DNA
atgaccagccccgtggagaacagcacctcaactgagaagctgaccctggcagagaaggtgtggcgcgaccatgtcgtgtccaagggagaaaacggcgagcccgacctcctctacatcgacctgcagctgctgcatgaagtgacctcaccacaggcatttgacggcctgcgcatgaccggccgtaaactgcgccacccagaactgcacctggccaccgaagaccacaacgtgccaaccgaaggcatcaagactggctcactgctggaaatcaacgacaagatttcccgcctgcaggtatctactctgcgcgacaactgtgaagaattcggcgtgcgcctgcacccaatgggtgatgtccgacagggcatcgtgcacaccgtcggcccacagctcggcgcaacccagccaggcatgaccattgtgtgcggtgactcccacacctccacccacggtgcttttggctccatggcattcggcatcggtacctcagaggttgagcacgtcatggctactcaaaccctgccactgaagcctttcaagaccatggccattgaagttactggtgaactgcagccaggtgtttcctccaaggacctgattctggcgattatcgccaagatcggcaccggcggcggacagggctacgttctggaataccgcggcgaagcaatccgtaagatgtccatggatgcacgcatgaccatgtgcaacatgtccatcgaagctggcgcacgtgccggcatgatcgccccagaccaaaccaccttcgactacgttgaaggccgcgaaatggcaccaaagggcgccgactgggacgaagcagttgcttactggaagaccctgccaaccgacgaaggcgcaacctttgacaaggtcgtagaaatcgatggctccgcactgaccccattcatcacctggggcaccaacccaggccagggcctgccactgggcgaatccgtaccaagcccagaagacttcaccaacgacaacgacaaggcagcagccgaaaaggcactgcagtacatggacctggtaccaggaaccccactgcgcgacatcaagatcgacaccgtcttcctgggatcctgcaccaacgcccgcatcgaagacctgcagatcgccgctgacatcctcaagggccacaaaatcgccgacggcatgcgcatgatggtcgtgccttcctccacctggatcaagcaagaggcagaagcgctcggactggacaaaatcttcaccgacgctggcgctgaatggcgtaccgcaggctgctccatgtgcctgggcatgaacccagaccaactgaagccaggcgagcgctccgcatccacctccaaccgaaacttcgaaggacgccaaggaccaggagaccgcacccacctggtatccccagcagtcgcagccgccaccgcaatccgcggcaccctgtcctcacctgcagatatctaa

SEQ ID NO: 34 - DNA, 2790 bp, synthetic construct
  misc_feature 1..2790: note = nucleotide variant of gene NCgl1432
  source 1..2790: mol_type = other DNA
atgagtttttctgccgaaaagggcacccacctttcagagttcatagcagacctgggctttgatctggacgagttccaaatcaaaggctgccacgctgtggaagaagaccacggtgttttagtatgtgcgcccaccggcgcgggcaaaacaattgttggtgaattcgcagtgtccctcgcattatcgcgggggacaaagtgtttctacaccacccccatcaaagcgctgagcaaccagaagtaccacgatttggtggctaaacacggctccgatgccgttggtctgctcaccggtgatgtttccattaaccatgatgctgacatcgtggtcatgaccaccgaagtgctgcgcaacatgatttacgcgggctcttttgcgcttgagcgcttaagccacgtggtcatggatgagatccacttccttgctgatgcctcccgtggcgcggtgtgggaagaagtgatcctcaacttggatgattccgtcaacatcatcggtctatctgccacggtgtccaactcagaggagtttggtgagtggctgaccactgttcgcggcgatacccgtgtgattgttactgatcaccgccccgttccgcttgatcagtacatgatggtgcagcgcaaagtgatgccactgtttgagcctggcaccgatggacgcgtgaacaaggagttagaggcaacgattgatcgcctcaacagcaagcaaagcgaacaaggccgtgcggcataccgctctggtgaaggcttccgtgcacgcagcaaaggcgataagcaggattctcgcactggtaagccacgggaacaagaccgccacaggccactgggtcggcctgaagtgctcagcatcctcaagggcatcaacatgctgccagcgattacgtttatcttctcccgcgcgggctgtgatggtgcgctgtaccaatgcttgcgttctaagttggtcttgacggatcaagcagaatcagaagagattgcacgcattgtcgacgccggcgtggtggggatccccgaggaagaccttcaagtactgaactttaagcagtggcgtgctgcactgatgcgcggtttcgcagcccaccacgcgggtatgcttccagcgtttaggcacatcgtggaagagctctttgttaaaggtcttgtccgcgcggtgtttgccacggaaaccctggcattgggaatcaacatgccagcgcgcaccgtggtgttggaaaagatggtcaaatttgacggcgaaggccacgttgatctcacccctggccaatacacgcagctgaccggtcgtgctggtcgacgtggcatcgatgtgttgggtaatgctgtggtgcagtggtcaccagcacttgatccacgatgggtggcaggtcttgcctctacgcgtacctacccgctgatctctacgttccagccgggctacaacatgtcggttaacctgctgaaaaccattggttatgagccttcgctgcgccttttggaaaaatcttttgcacagttccaagccgatggttccgtcgtgggcgatgtgcgtgaaattgaacgtgcagaagccaaggtggcagaattgcgtgcccagctgaacaaagagattgctgccaccaaccctgcggtgcgtgaagatcaagacgcagtggaggtgtttatcgactacatggagcttcgccgtgagctcaatgaggaagaaaaactcaatcgcaagcaaagcatcgaagatcgcaacgtagaaacagtccgtgtgctgtccaagctgcaaatcggtgatgtcattgccatgcctggtagaaaacgaccagttctcgcagtagtgatgacgcctgctaatcagagcagagatccccgcccatgggtgaccaccgaatctggttggtcaggtcgtgtggatgcggaatcctttactaatccgccgatcaccattgggcatatgcgtctgcctcgccaagctattgaagagcctcgccgcaatgcccggcgcgtccaggaactgtttaggcgtgagcacttcaagcgacccaacaagatgcgggagtttgctcgggttcgtcccaatgaggcagtgaccaaactgcgtaatgctattcgggatcatgaggcgtatcattggcctgatcgggagcacttggctcgcaccgcggagcgtatgatccgtaaagaacgtgatctggctaagttgaccggcaatgtggataaagccagggaaaccctcggtaggacgtttgagcgcattttgtcgctgctcagtgaaatggactatgtggattactctaatccagataatccagtgatcactgatgaaggtgagcgtttggcgaaaatccacagtgaggcagacctgttggttgctcagtgcctcaagcgtggcatttgggacaaccttgatcccgcagagctcgccggtgtggtgagtatgtgcacgtttgaaaatcgtcgcgaaaccggtggtgaggctcaagctgtcacagaggccatggctgattccatgaatagcgtggaacgtatttggggtgagctggttgaagatgagcgccgtcaccgtctgccaattactcgccagccggaagcaggttttgccaccgcgatccaccagtgggcttcaggtgctccgctgggatattgcatggctgcggcagcggaaaacggcgcggagttgacccctggtgacttcgtgcgctggtgccgtcaagtcatcgatcttctagagcaggttgctaagactgcctactttgatgagaccacacggaatgctcgtcaggctattgatgcgattaggcgtggagttgtggcgatcggttcctag

SEQ ID NO: 35 - DNA, 582 bp, synthetic construct
  misc_feature 1..582: note = nucleotide variant of gene NCgl1531
  source 1..582: mol_type = other DNA
gtgacaaccaacgcccccgacggagcaacgaacaacatcaacaacgcacattcgggcgctgtcgggaagccaaaggtacagctcagcgatgcggaaattcagaaatacaccgcagctttcgctggcaccaccacaaccaagccatgggagctggaggtgaccacaaagtttctgaaaaagatcgcgtgggtagccgtggttgtcatcatggccgttcacatcttcatgggtgccgtggtggacgtcgatttcaccggtgcagcggtcacctttgttgacactctggcattcccagcgttgggcatcatcttctccgttcttgtgttcttgggactgactcgccctcgcgtgcgtgccaacgaagacggcgttgaggtgcgtaacttcatcggaactcgtttctacccatgggttgtcatctacggcatgtctttccccaagggcagcagcgtggcacgtttggagcttccagactttgaattcgttcccatgtgggctttccagtcccgcgatggagaagatgtggtgcgcgcggttgcgaccttccgcgacctcgaaaacaagtacatgccagaggactaa

SEQ ID NO: 36 - DNA, 558 bp, synthetic construct
  misc_feature 1..558: note = nucleotide variant of gene NCgl1588
  source 1..558: mol_type = other DNA
atgaagcttttctcccgcacctcactggttgcacttggtaccgctgcagctatcactctctccggcgtaaccgctcctgcattcgctgatgaggactccaacgcagctgtaagtgctcttaagaccgctgaagataatacccctgaggcgccaggggcttctactcccctgaagcttgagcagcctggcaccatcaccggcgtccctggcaaggcgatcaccccggtcactgttaaggtcatcgcaggcgaagcagaatccttcacctcagacaaccttccttctggtctccttatcgacaacaccggaaagatcaccggtactccaaagaaggaattcactggttccgcaaagatcattgccaagaacgaagcaggcgttgaagcagaagtttacgttaactttgatttcaacgaagagccttccagcgaagagccttccagcggttcttccgacactgacaacatcgaaaactggatcaagatcatcacagcagtcatcggtgcactaaccaccattttaaccttcagtaccaagctggattccttcctgaagtaa

SEQ ID NO: 37 - DNA, 795 bp, synthetic construct
  misc_feature 1..795: note = nucleotide variant of gene NCgl1859
  source 1..795: mol_type = other DNA
atggtcagccaaacggaaagacagcatgcaattgcttctttactggcaccaactggtgcggtgtctgtaggagatttagccgagcatttccatgtgacaaccgaaacagtgcgacgtgatcttcggatcatggagtcactgggtttgttgcaacgagttcacggtggcgccattagcccagagcccatgggtacgtctccccctcggctgaaacctgccttggttaaaggaatgccaccggaaccccgtgttttagaacttgcagaaactgcagtttccctcatcacacctctagcacgcagcattttcctggattcaggtttagcgtgcacggcgattgccacggtgttgggggatcctccagaagatgccaggtggactgttgttacaagttcccccggcgctgtgattgccttgtccgcgacagatgccacctccacggtggtgctgcacgggcaggttcacggtaattgttcttcaatcattgggtccacggcagtagacatgatttcgcagttgcgcgctgatatcgccttcgtggaggttgatgcgattcaatccgatacaagtctgtgcacgtttttcccggagacgattcccatcaagcaagccatgatcaaaaacgcggctttcacagttgctgttctcagcccgagatctccccaagatcaagaacttcaacttttgaagcaccctttttccaccttggctgattttgatgcccttgttaccgatgaccacacgctagattttccagttttgcccgaccacaactttcaggtggtaaccccatga

SEQ ID NO: 38 - DNA, 1581 bp, synthetic construct
  misc_feature 1..1581: note = nucleotide variant of gene NCgl1874
  source 1..1581: mol_type = other DNA
gtgacgcagcaattgaaccacgcaaaggtaaatcaacatcccggtcaagccaccctcccagaaaccgcagaggggcaggttcgcacctacgaggtaaaaacctacggctgtcagatgaatgtgcacgattctgagcgcctttcgggcctgctcgaggaggctggatacgttgctgctccggaggacaccactccggatcttgtcgtatttaatacgtgcgccgtgcgtgaaaacgccgatatgcgcctctatggcactttgggcaacctgcgcagcgtgaaagaaaagaacccaggcatgcaaatcgctgtcggtggttgtttggctcaaaaagacaaagataccgtggtgaaaaaagcaccgtgggtggacgtggtgtttggtacccacaacattggttccttgccaaccttgcttcagcgcgcggagcacaatgcccaagcggaagtcgaaattgtcgattccctcgagcagttcccgtcagtacttcctgcaaagcgcgagtctgcttacgctggttgggtgtccgtatcagtcggatgtaacaacacctgtactttctgcatcgttccgtcgctgcgcggtaaagagcaggaccgtcgaccaggagacatcctcgcagaggtacaagcactggtggatcagggagttaccgaggtaactctacttggccaaaacgtaaatgcttacggcgtgaactttgttgatcctgagctagagcgcgatcgcagtgcattttccaagctgcttcgtgcctgtggtgagatcgaaggcctcgagcgggttcgcttcaccagccctcaccctgcagaattcacctctgatgtcattgacgccatggcagagaccccaaacatctgcccgcagctgcacatgccactgcagtccggatctgacaaggtgctcaaagagatgcgccgttcctaccgatccaagaagttcctctccatcttggatgaggtccgtgcgaagatccctcacgcctctatcaccaccgatattattgtcggattccctggcgaaacagaggaggatttccaagcaaccctcgacgttgtcaagaaggcacgctttacttctgcttacaccttccaatacagcccacgccctggcacccctgcagcggaatatgaaaaccagcttccaaaagaagttgtgcaggaacgctacgagcgcctcatggtcgttcaggaacaagtctgcgaagaagaaaaccaaaagctcatcggcaccaccgtcgaattgctggtccaggctggcggaggccgcaagaacgatgccaccaagcgcatgagtggtcgcgcacgcgatggacgcctcgtgcactttgcgccagagggcgacattgatggtgagatccgccccggcgattttgtcactgtcacggtgactgaggccaagcctttcttcctcatcgcagactccggtgtgcagacccaccgccgcaccaaagctggtgacaactctgcagttggtcaagttccaaccacagcaccgatcggtgtgggcttgggactgccacaaatcggcgcaccaaaggtggctcctgccacagaatctgcctgctgctccattaactaa

SEQ ID NO: 39 - DNA, 117 bp, synthetic construct
  misc_feature 1..117: note = nucleotide variant of gene NCgl3069
  source 1..117: mol_type = other DNA
gtggctgtcgcaaaagacgtgcttagtttttcacgacccattcccgcacttcacgccatcatcggcgcgcttggatggtttggaatgttcgcagttagtctgtggagcacgctgtaa

SEQ ID NO: 40 - DNA, 1554 bp, synthetic construct
  misc_feature 1..1554: note = nucleotide variant of gene NCgl2356
  source 1..1554: mol_type = other DNA
atgagcatcaccacacacgtccaagcactcaccacagcactcaacgccatcgacaaccatttggccagcatgctcgaccatggtgtcaccccagaccaatacaaggccatcgagcccgacctcatcgccctagaacacaccatcaaccaccacgccaccatcgccgcccaaaccacagccctcgccgaacgcaccaacgccgcccacaccattggctccacccacctcatcgactacctcaccaccaccttcggactatccaaagcacgcgcccaccaccgcatcaatctcgcccactccctctaccccataccgaagccaaaccctggatctggcaacggcggtaatggtggcaatcccgacggtggtcctgatggtggcgactcgggtgatgacgactccggcgacgatgaccccgaccccgaaccggacaagcctgaagacggcaaacctgatggtgataagcctcgtgggccacggatcagcgcggaaaaacacgccatcatcaccgacgaactcgcccgcctcaacccgaataccacacccagcgccgaggagctacgcacccaagccctgagtcaagcgatctggcgcaccccagaagacctccgcacgtggctacgccaccacgtcaccaccgccaacaaaaacaaccccaaccccatcaccgccatgaaaaggcgctacctcgctgtaggtaaacccgatgccgacaacatggtccgcatcagcggcctcgtgcccgcagccaccgcagcactgatcaccgcgaacaccgcaccgttaaccaaacgcggcaacctcgtggatctacccgcagcagaagatatgcgcacccgcgggcaacgccatgcggacgcgttgcatcacatcatggagatctacaaccacggtattgtcaccccagctcgtggtggaacagccagcatcatcatctccatgaccaccgatgatcttgatgagatcaaccacggtgatcatggcgatggcagtctacttaacaacctgtaccccaccaatacgggttactcattgaacttggcggagatcatgaacctcatcgctgcgaaatacgacttcgctgtgctcctcgatggtgagacggggcagccgttgaacgtcaataggatgcagcgctcagcgaacctgactcaacgcatcgcgttgtttgcttctgagttggtgtgctcggcacccaattgtgacaggccgcagttagagtgcgaggttcatcatttagatccctggatgagaggtgggctgaccaacctggtcaatctcacgcatcagtgctttaatcaccacccacgcaacgatgattccaggagtggggtcaatggtaaagggtttatggaccgcgatcctgctactggaagagtggggcactacccagtgggtggtgaggggccggtgtttaaccggtcggctgctgctgatcgttccggtggtgcgtgggcgaggcgtaagcatcatggcccgccacccacaccgccggacccgccggatccgcctggtcctgagccggatcctggtgatgagggcagattgttctag

SEQ ID NO: 41 - DNA, 126 bp, synthetic construct
  misc_feature 1..126: note = nucleotide variant of gene NCgl3082
  source 1..126: mol_type = other DNA
gtgcgtatgttgtttgagaactcaatagtgtgccatttattatttttgtcactaccacagatcaccttgggtgatgtgtggtgggtcatgccgggtggtggatcgccaaattatcgatcactgtaa

SEQ ID NO: 42 - DNA, 1446 bp, synthetic construct
  misc_feature 1..1446: note = nucleotide variant of gene NCgl2542
  source 1..1446: mol_type = other DNA
atgcctaaacccctacccccagaaacccgacgcaagatcatcgatttcgatccgttcgcaccgaacagcccctcgatcgaagagttctgcagtcggctaaaaatatcgcggcgcagcttctacaacatccgcaaccgataccaacaagacgccaacgcagcactgcatccacactccagcgccccaatcaccgcccggcgaacgtacgatgaatccatcaccagcaccttgctgtccatccgcgcacgcctgaaagcccaaggatgggagtacggcccgatctctattcgattcgaaggcatctccaccggggaactgactgcaccgattccatctgtttcaaccattgctcgtttgttacgcgccgcaggagctgttgaaagtaaccctaagaagcgaccgaagtcgtcggtggtgaggtttcaacgaggtcaagccatggaaatgtggcaaatagatggtttcatctacacactgcacgatactgatctgactcgggtaacgatctatcaaatccttgatgatgccactcggtttgatgtcggaacctgtgtcttccccgcgaatgaaaactcagtcgatgcccgaacagcgctagaacaagcgattgctcatttcggtgccccgcatgaattactcagtgataacggctcagcgtttaaccggatgcggcaaggatacgtcggaagcttggaaagctatctcgcgacggtggggtgtttaagcattaccggcaagcctgggcatcctcaaacccaaggtaaaaacgaacgcagccaccgcacactatttcgtttccttcaagctcatcaaccacacacacttgaggaatgtgcgcactatattgaacagttccgcgatcattacaacaatcgtcgcccgcatcaggggttgccgaataatctctccccggccgcggcctgggagattgtgggctgtgtggaacaacaacccccgattgatcccgtcgtgcttcaacagcaagccgatcactatgcccgtcgtcgaattgagaagcaatcagatgtcccgcttgttcggcaggaggaatctgttccggtgtctaagatgcagcagaccgagcaacgtcgacgggtacgtcgttttggtaaaaagccggtggatcctgatgtgtttacgtttgctgggaataatcagaaggtggtgttccaggggatgcgtatttctgttcctcgtacgatgagggacagggagttttatcggacggtgacggcaactgagcttggtttctgggatgcgataaccggggagcttgagttgtcgattccgttgccggttgtggcgattgcccggggtaagtcgtatatcaattcttacaacattcgtggggtgtggatgcaacacccgacaccgttgtggcaacgcaaacgtgatgaggctgagaagcgattcaagtcgatagatccgggggatcttctgcgctag

SEQ ID NO: 43 - DNA, 1833 bp, synthetic construct
  misc_feature 1..1833: note = nucleotide variant of gene NCgl2765
  source 1..1833: mol_type = other DNA
atgactactgctgcaatcaggggccttcagggcgaggcgccgaccaagaataaggaactgctgaactggatcgcagacgccgtcgagctcttccagcctgaggctgttgtgttcgttgatggatcccaggctgagtgggatcgcatggcggaggatcttgttgaagccggtaccctcatcaagctcaacgaggaaaagcgtccgaacagctacctagctcgttccaacccatctgacgttgcgcgcgttgagtcccgcaccttcatctgctccgagaaggaagaagatgctggcccaaccaacaactgggctccaccacaggcaatgaaggacgaaatgtccaagcattacgctggttccatgaaggggcgcaccatgtacgtcgtgcctttctgcatgggtccaatcagcgatccggaccctaagcttggtgtgcagctcactgactccgagtacgttgtcatgtccatgcgcatcatgacccgcatgggtattgaagcgctggacaagatcggcgcgaacggcagcttcgtcaggtgcctccactccgttggtgctcctttggagccaggccaggaagacgttgcatggccttgcaacgacaccaagtacatcacccagttcccagagaccaaggaaatttggtcctacggttccggctacggcggaaacgcaatcctggcaaagaagtgctacgcactgcgtatcgcatctgtcatggctcgcgaagaaggatggatggctgagcacatgctcatcctgaagctgatcaacccagagggcaaggcgtaccacatcgcagcagcattcccatctgcttgtggcaagaccaacctcgccatgatcactccaaccatcccaggctggaccgctcaggttgttggcgacgacatcgcttggctgaagctgcgcgaggacggcctctacgcagttaacccagaaaatggtttcttcggtgttgctccaggcaccaactacgcatccaacccaatcgcgatgaagaccatggaaccaggcaacaccctgttcaccaacgtggcactcaccgacgacggcgacatctggtgggaaggcatggacggcgacgccccagctcacctcattgactggatgggcaacgactggacctcagagtccgacgaaaacgctgctcaccctaactcccgttactgcgtagcaatcgaccagtccccagcagcagcacctgagttcaacgactgggaaggcgtcaagatcgacgcaatcctcttcggtggacgtcgcgcagacaccgtcccactggttacccagacctacgactgggagcacggcaccatggttggtgcactgctcgcatccggtcagaccgcagcttccgcagaagcaaaggtcggcacactccgccacgacccaatggcaatgctcccattcattggctacaacgctggtgaatacctgcagaactggattgacatgggtaacaagggtggcgacaagatgccatccatcttcctggtcaactggttccgccgtggcgaagatggacgcttcctgtggcctggcttcggcgacaactctcgcgttctgaagtgggtcatcgaccgcatcgaaggccacgttggcgcagacgagaccgttgttggacacaccgctaaggccgaagacctcgacctcgacggcctcgacaccccaattgaggatgtcaaggaagcactgaccgctcctgcagagcagtgggcaaacgacgttgaagacaacgccgagtacctcactttcctcggaccacgtgttcctgcagaggttcacagccagttcgatgctctgaaggcccgcatttcagcagctcacgcttaa

SEQ ID NO: 44 - DNA, 1302 bp, synthetic construct
  misc_feature 1..1302: note = nucleotide variant of gene NCgl2816??
  source 1..1302: mol_type = other DNA
atgacaaccgcagtagatcaaaactcaccgcccaagcagcaactcaacaagcgcgtcctgctgggcagcttgagtggcagcgttatcgaatggttcgacttcctggtttacggaaccgtcgccgcgctggtcttcaacaagatgtacttccccagcggcaacgagttcctctccacaatcctggcgtacgcatccttctccctgaccttcttcttccgccccattggtggcgtcatcttcgcccacatcggcgaccgcattgggcgtaagaagaccctgttcatcaccttgatgctcatgggtggcggcaccgtcgccattggtttgctgcccgactacaacgccatcggcatttgggcaccaatccttctgatgttcctccgcattttgcagggcatcggaattggcggcgaatggggtggcgcactgctcctggcatacgaatacgctccaaagaagcagcgtgggctctacggcgcagttcctcaaatgggcatttccctgggcatgctgcttgcagctggcgtgatctctctgctcaccctcatgccggaagatcagttcctcacctggggctggcgcatcccattcgtcggatccatcctcctagtgttcatcggcctgttcatccgaaacggccttgatgaaacccccgagtgcaagcgtatccgcgattccggccagcaggtaaagatgcctctgaaggaagttctgaccaagtactggccagccgttctggtctccatcggcgcaaaagctgccgagaccggccccttctacatcttcggcacctacatcgttgcttacgcaaccaacttcctgaacatccgcgacaacattgtccttctggcagttgcttgcgccgccctcgttgccaccatctggatgccactgttcggatccttctccgaccgcgtcaaccgtgcagtgctctacaggatctgtgcatccgcaaccatcgtgctgattgtcccttactacttggtcctcaacaccggcgaaatttgggcactgtttatcactaccgtgattggcttcggcatcctctggggtagcgtcaacgcaatcctcggaaccgtcatcgcagaaaacttcgcacctgaggtccgctacaccggcgctaccctgggttaccaagtcggagcagcactcttcggcggtaccgcacccattatcgcagcatggctgttcgaaatctccggcggacaatggtggccaatcgccgtctacgtcgctgcatgttgccttctctctgtgatcgcctcgttcttcatccaacgcgtcgcgcaccaagagaactaa

SEQ ID NO: 45 - DNA, 40 bp, synthetic construct
  misc_feature 1..40: note = NCgl0030*_F
  source 1..40: mol_type = other DNA
tgaattcgagctcggtaccccctgctgatgatcgctgatg

SEQ ID NO: 46 - DNA, 39 bp, synthetic construct
  misc_feature 1..39: note = NCgl0030*_R
  source 1..39: mol_type = other DNA
tcgactctagaggatcccccattccaaagatgagtgcac

SEQ ID NO: 47 - DNA, 40 bp, synthetic construct
  misc_feature 1..40: note = NCgl0288*_F
  source 1..40: mol_type = other DNA
tgaattcgagctcggtaccccaaaaagcatcagcaagagc

SEQ ID NO: 48 - DNA, 39 bp, synthetic construct
  misc_feature 1..39: note = NCgl0288*_R
  source 1..39: mol_type = other DNA
tcgactctagaggatccccatgtgaaaacatggtccact

SEQ ID NO: 49 - DNA, 40 bp, synthetic construct
  misc_feature 1..40: note = NCgl0337*_F
  source 1..40: mol_type = other DNA
tgaattcgagctcggtaccctttcgtgcgttacgtactaa

SEQ ID NO: 50 - DNA, 39 bp, synthetic construct
  misc_feature 1..39: note = NCgl0337*_R
  source 1..39: mol_type = other DNA
tcgactctagaggatccccgctattgctcattgttggcc

SEQ ID NO: 51 - DNA, 40 bp, synthetic construct
  misc_feature 1..40: note = NCgl0458*_F
  source 1..40: mol_type = other DNA
tgaattcgagctcggtaccccacttggtgacaccgatgag

SEQ ID NO: 52 - DNA, 39 bp, synthetic construct
  misc_feature 1..39: note = NCgl0458*_R
  source 1..39: mol_type = other DNA
tcgactctagaggatcccctaagtggtgcagtttagcta

SEQ ID NO: 53 - DNA, 40 bp, synthetic construct
  misc_feature 1..40: note = NCgl0686*_F
  source 1..40: mol_type = other DNA
tgaattcgagctcggtacccccacgcattatttccggaca

SEQ ID NO: 54 - DNA, 39 bp, synthetic construct
  misc_feature 1..39: note = NCgl0686*_R
  source 1..39: mol_type = other DNA
tcgactctagaggatccccccagaccactggaacgctga

SEQ ID NO: 55 - DNA, 40 bp, synthetic construct
  misc_feature 1..40: note = NCgl0706*_F
  source 1..40: mol_type = other DNA
tgaattcgagctcggtaccccgtggctacttctgcgatcc

SEQ ID NO: 56 - DNA, 39 bp, synthetic construct
  misc_feature 1..39: note = NCgl0706*_R
  source 1..39: mol_type = other DNA
tcgactctagaggatccccgtgcggcccctgcaaaatgg

SEQ ID NO: 57 - DNA, 40 bp, synthetic construct
  misc_feature 1..40: note = NCgl0799*_F
  source 1..40: mol_type = other DNA
tgaattcgagctcggtaccccgccagaagatggaaggtta

SEQ ID NO: 58 - DNA, 39 bp, synthetic construct
  misc_feature 1..39: note = NCgl0799*_R
  source 1..39: mol_type = other DNA
tcgactctagaggatccccggccaccagacaccttgacg

SEQ ID NO: 59 - DNA, 40 bp, synthetic construct
  misc_feature 1..40: note = NCgl1165*_F
  source 1..40: mol_type = other DNA
tgaattcgagctcggtacccattgcttccaagggtattta

SEQ ID NO: 60 - DNA, 39 bp, synthetic construct
  misc_feature 1..39: note = NCgl1165*_R
  source 1..39: mol_type = other DNA
tcgactctagaggatcccctcaacctcattcgcccagac

SEQ ID NO: 61 - DNA, 40 bp, synthetic construct
  misc_feature 1..40: note = NCgl1262*_F
  source 1..40: mol_type = other DNA
tgaattcgagctcggtacccaccccactgcgcgacatcaa

SEQ ID NO: 62 - DNA, 39 bp, synthetic construct
  misc_feature 1..39: note = NCgl1262*_R
  source 1..39: mol_type = other DNA
tcgactctagaggatccccgacagcgcggaagccgtagt

SEQ ID NO: 63 - DNA, 40 bp, synthetic construct
  misc_feature 1..40: note = NCgl1432*_F
  source 1..40: mol_type = other DNA
tgaattcgagctcggtacccatgcctggtagaaaacgacc

SEQ ID NO: 64 - DNA, 39 bp, synthetic construct
  misc_feature 1..39: note = NCgl1432*_R
  source 1..39: mol_type = other DNA
tcgactctagaggatcccctcagccatggcctctgtgac

SEQ ID NO: 65 - DNA, 40 bp, synthetic construct
  misc_feature 1..40: note = NCgl1531*_F
  source 1..40: mol_type = other DNA
tgaattcgagctcggtacccgctcttgatacttccacccc

SEQ ID NO: 66 - DNA, 39 bp, synthetic construct
  misc_feature 1..39: note = NCgl1531*_R
  source 1..39: mol_type = other DNA
tcgactctagaggatccccttggggaaagacatgccgta

SEQ ID NO: 67 - DNA, 40 bp, synthetic construct
  misc_feature 1..40: note = NCgl1588*_F
  source 1..40: mol_type = other DNA
tgaattcgagctcggtacccttaaataacatcttgcttga

SEQ ID NO: 68 - DNA, 39 bp, synthetic construct
  misc_feature 1..39: note = NCgl1588*_R
  source 1..39: mol_type = other DNA
tcgactctagaggatccccgattcacaaaggattagtcg

SEQ ID NO: 69 - DNA, 40 bp, synthetic construct
  misc_feature 1..40: note = NCgl1859*_F
  source 1..40: mol_type = other DNA
tgaattcgagctcggtaccccacttttaataacttcatac

SEQ ID NO: 70 - DNA, 39 bp, synthetic construct
  misc_feature 1..39: note = NCgl1859*_R
  source 1..39: mol_type = other DNA
tcgactctagaggatcccccagacttgtatcggattgaa

SEQ ID NO: 71 - DNA, 40 bp, synthetic construct
  misc_feature 1..40: note = NCgl1874*_F
  source 1..40: mol_type = other DNA
tgaattcgagctcggtacccgcgcctttcgggcctgctcg

SEQ ID NO: 72 - DNA, 39 bp, synthetic construct
  misc_feature 1..39: note = NCgl1874*_R
  source 1..39: mol_type = other DNA
tcgactctagaggatccccgtcaatgacatcagaggtga

SEQ ID NO: 73 - DNA, 40 bp, synthetic construct
  misc_feature 1..40: note = NCgl2356*_F
  source 1..40: mol_type = other DNA
tgaattcgagctcggtacccgttgcatcacatcatggaga

SEQ ID NO: 74 - DNA, 39 bp, synthetic construct
  misc_feature 1..39: note = NCgl2356*_R
  source 1..39: mol_type = other DNA
tcgactctagaggatcccctaccgaacgggccggagccg

SEQ ID NO: 75 - DNA, 20 bp, synthetic construct
  misc_feature 1..20: note = NCgl0030_F
  source 1..20: mol_type = other DNA
ggcgccgtgcttgtttttac

SEQ ID NO: 76 - DNA, 20 bp, synthetic construct
  misc_feature 1..20: note = NCgl0030_R
  source 1..20: mol_type = other DNA
atcgctccttgttgaaacgc

SEQ ID NO: 77 - DNA, 20 bp, synthetic construct
  misc_feature 1..20: note = NCgl0288_F
  source 1..20: mol_type = other DNA
cctgcacgtcaccgtcattt

SEQ ID NO: 78 - DNA, 20 bp, synthetic construct
  misc_feature 1..20: note = NCgl0288_R
  source 1..20: mol_type = other DNA
gcctcaaatggatctgacgg

SEQ ID NO: 79 - DNA, 20 bp, synthetic construct
  misc_feature 1..20: note = NCgl0337_F
  source 1..20: mol_type = other DNA
ttgcgcgatattgaagaggt

SEQ ID NO: 80 - DNA, 20 bp, synthetic construct
  misc_feature 1..20: note = NCgl0337_R
  source 1..20: mol_type = other DNA
gcccccggaagctcaagttc

SEQ ID NO: 81 - DNA, 20 bp, synthetic construct
  misc_feature 1..20: note = NCgl0458_F
  source 1..20: mol_type = other DNA
ctggaagaagagaccctaga

SEQ ID NO: 82 - DNA, 20 bp, synthetic construct
  misc_feature 1..20: note = NCgl0458_R
  source 1..20: mol_type = other DNA
ctgatctttacgtaaccggg

SEQ ID NO: 83 - DNA, 20 bp, synthetic construct
  misc_feature 1..20: note = NCgl0686_F
  source 1..20: mol_type = other DNA
ccccagaagcacccgttgtg

SEQ ID NO: 84 - DNA, 20 bp, synthetic construct
  misc_feature 1..20: note = NCgl0686_R
  source 1..20: mol_type = other DNA
cgccattggccacatccaag

SEQ ID NO: 85 - DNA, 21 bp, synthetic construct
  misc_feature 1..21: note = NCgl0706_F
  source 1..21: mol_type = other DNA
gatctgcttgctgaacatgat

SEQ ID NO: 86 - DNA, 20 bp, synthetic construct
  misc_feature 1..20: note = NCgl0706_R
  source 1..20: mol_type = other DNA
tcataagtgggctttgtttg

SEQ ID NO: 87 - DNA, 20 bp, synthetic construct
  misc_feature 1..20: note = NCgl0799_F
  source 1..20: mol_type = other DNA
gtctacgttctggttgcatc

SEQ ID NO: 88 - DNA, 20 bp, synthetic construct
  misc_feature 1..20: note = NCgl0799_R
  source 1..20: mol_type = other DNA
agctgagtggtcagagttgc

SEQ ID NO: 89 - DNA, 20 bp, synthetic construct
  misc_feature 1..20: note = NCgl1165_F
  source 1..20: mol_type = other DNA
ttaccagccaaccctggctg

SEQ ID NO: 90 - DNA, 20 bp, synthetic construct
  misc_feature 1..20: note = NCgl1165_R
  source 1..20: mol_type = other DNA
actacttcagctaaacggag

SEQ ID NO: 91 - DNA, 20 bp, synthetic construct
  misc_feature 1..20: note = NCgl1262_F
  source 1..20: mol_type = other DNA
aatcgatggctccgcactga

SEQ ID NO: 92 - DNA, 20 bp, synthetic construct
  misc_feature 1..20: note = NCgl1262_R
  source 1..20: mol_type = other DNA
acagaagttcgatgtcggac

SEQ ID NO: 93 - DNA, 20 bp, synthetic construct
  misc_feature 1..20: note = NCgl1432_F
  source 1..20: mol_type = other DNA
gcgtgaagatcaagacgcag

SEQ ID NO: 94 - DNA, 20 bp, synthetic construct
  misc_feature 1..20: note = NCgl1432_R
  source 1..20: mol_type = other DNA
ctggtggatcgcggtggcaa

SEQ ID NO: 95 - DNA, 20 bp, synthetic construct
  misc_feature 1..20: note = NCgl1531_F
  source 1..20: mol_type = other DNA
gtagtgcaagaactggcacg

SEQ ID NO: 96 - DNA, 20 bp, synthetic construct
  misc_feature 1..20: note = NCgl1531_R
  source 1..20: mol_type = other DNA
cgcaccacatcttctccatc

SEQ ID NO: 97 - DNA, 20 bp, synthetic construct
  misc_feature 1..20: note = NCgl1588_F
  source 1..20: mol_type = other DNA
gcaggcaataggtagtaaat

SEQ ID NO: 98 - DNA, 20 bp, synthetic construct
  misc_feature 1..20: note = NCgl1588_R
  source 1..20: mol_type = other DNA
cttaggtttaaatattcgaa

SEQ ID NO: 99 - DNA, 20 bp, synthetic construct
  misc_feature 1..20: note = NCgl1859_F
  source 1..20: mol_type = other DNA
aagcgatcaccatatttcat

SEQ ID NO: 100 - DNA, 20 bp, synthetic construct
  misc_feature 1..20: note = NCgl1859_R
  source 1..20: mol_type = other DNA
gggcatcaaaatcagccaag

SEQ ID NO: 101 - DNA, 20 bp, synthetic construct
  misc_feature 1..20: note = NCgl1874_F
  source 1..20: mol_type = other DNA
ataggcgtttatgtcagctc

SEQ ID NO: 102 - DNA, 20 bp, synthetic construct
  misc_feature 1..20: note = NCgl1874_R
  source 1..20: mol_type = other DNA
gggatcttcgcacggacctc

SEQ ID NO: 103 - DNA, 20 bp, synthetic construct
  misc_feature 1..20: note = NCgl2356_F
  source 1..20: mol_type = other DNA
caaccccatcaccgccatga

SEQ ID NO: 104 - DNA, 20 bp, synthetic construct
  misc_feature 1..20: note = NCgl2356_R
  source 1..20: mol_type = other DNA
caccggtgaaaaggagagaa

SEQ ID NO: 105 - protein, 264 aa, synthetic construct
  REGION 1..264: note = Wild type protein of gene NCgl1859
MVSQTERQHAIASLLAPTGAVSVGDLAEHFHVTTETVRRDLRIMESLGLLQRVHGGAISPEPMGTSPPRLKPALGKGMPPEPRVLELAETAVSLITPLARSIFLDSGLACTAIATVLGDPPEDARWTVVTSSPGAVIALSATDATSTVVLHGQVHGNCSSIIGSTAVDMISQLRADIAFVEVDAIQSDTSLCTFFPETIPIKQAMIKNAAFTVAVLSPRSPQDQELQLLKHPFSTLADFDALVTDDHTLDFPVLPDHNFQVVTP

SEQ ID NO: 106 - protein, 193 aa, synthetic construct
  REGION 1..193: note = Wild type protein of gene NCgl1531
MTTNAPDGATNNINNAHSGAVGKPKVQLSDAEIQEYTAAFAGTTTTKPWELEVTTKFLKKIAWVAVVVIMAVHIFMGAVVDVDFTGAAVTFVDTLAFPALGIIFSVLVFLGLTRPRVRANEDGVEVRNFIGTRFYPWVVIYGMSFPKGSSVARLELPDFEFVPMWAFQSRDGEDVVRAVATFRDLENKYMPED

SEQ ID NO: 107 - DNA, 5802 bp, synthetic construct
  misc_feature 1..5802: note = pDC24 vector
  source 1..5802: mol_type = other DNA
gttcgcttgctgtccataaaaccgcccagtctagctatcgccatgtaagcccactgcaagctacctgctttctctttgcgcttgcgttttcccttgtccagatagcccagtagctgacattcatccggggtcagcaccgtttctgcggactggctttctacgtgttccgcttcctttagcagcccttgcgccctgagtgcttgcggcagcgtgaagctagcttttatcgccattcgccattcaggctgcgcaactgttgggaagggcgatcggtgcgggcctcttcgctattacgccagctggcgaaagggggatgtgctgcaaggcgattaagttgggtaacgccagggttttcccagtcacgacgttgtaaaacgacggccagtgaattcgagctcggtacccggggatcctctagagtcgacctgcaggcatgcaagcttggcgtaatcatggtcatagctgtttcctgtgtgaaattgttatccgctcacaattccacacaacatacgagccggaagcataaagtgtaaagcctggggtgcctaatgagtgagctaactcacattaattgcgttgcgctcactgcccgctttccagtcgggaaacctgtcgtgccagctgcattaatgaatcggccaacgcgcggggagaggcggtttgcgtattgggcgctcttccgcttcctcgctcactgactcgctgcgctcggtcgttcggctgcggcgagcggtatcagctcactcaaaggcggtaatacggttatccacagaatcaggggataacgcaggaaagaacatgtgagcaaaaggccagcaaaaggccaggaaccgtaaaaaggccgcgttgctggcgtttttccataggctccgcccccctgacgagcatcacaaaaatcgacgctcaagtcagaggtggcgaaacccgacaggactataaagataccaggcgtttccccctggaagctccctcgtgcgctctcctgttccgaccctgccgcttaccggatacctgtccgcctttctcccttcgggaagcgtggcgctttctcaatgctcacgctgtaggtatctcagttcggtgtaggtcgttcgctccaagctgggctgtgtgcacgaaccccccgttcagcccgaccgctgcgccttatccggtaactatcgtcttgagtccaacccggtaagacacgacttatcgccactggcagcagccactggtaacaggattagcagagcgaggtatgtaggcggtgctacagagttcttgaagtggtggcctaactacggctacactagaaggacagtatttggtatctgcgctctgctgaagccagttaccttcggaaaaagagttggtagctcttgatccggcaaacaaaccaccgctggtagcggtggtttttttgtttgcaagcagcagattacgcgcagaaaaaaaggatctcaagaagatcctttgatcttttctacggggtctgacgctcagtggaacgaaaactcacgttaagggattttggtcatgagattatcaaaaaggatcttcacctagatccttttggggtgggcgaagaactccagcatgagatccccgcgctggaggatcatccagccctgatagaaacagaagccactggagcacctcaaaaacaccatcatacactaaatcagtaagttggcagcatcacccgacgcactttgcgccgaataaatacctgtgacggaagatcacttcgcagaataaataaatcctggtgtccctgttgataccgggaagccctgggccaacttttggcgaaaatgagacgttgatcggcacgtaagaggttccaactttcaccataatgaaataagatcactaccgggcgtattttttgagttatcgagattttcaggagctgatagaaacagaagccactggagcacctcaaaaacaccatcatacactaaatcagtaagttggcagcatcacccgacgcactttgcgccgaataaatacctgtgacggaagatcacttcgcagaataaataaatcctggtgtccctgttgataccgggaagccctgggccaacttttggcgaaaatgagacgttgatcggcacgtaagaggttccaactttcaccataatgaaataagatcactaccgggcgtattttttgagttatcgagattttcaggagctctttggcatcgtctctcgcctgtcccctcagttcagtaatttcctgcatttgcctgtttccagtcggtagatattccacaaaacagcagggaagcagcgcttttccgctgcataaccctgcttcggggtcattatagcgattttttcggtatatccatcctttttcgcacgatatacaggattttgccaaagggttcgtgtagactttccttggtgtatccaacggcgtcagccgggcaggataggtgaagtaggcccacccgcgagcgggtgttccttcttcactgtcccttattcgcacctggcggtgctcaacgggaatcctgctctgcgaggctggccggctaccgccggcgtaacagatgagggcaagcggatggctgatgaaaccaagccaaccaggaagggcagcccacctatcaaggtgtactgccttccagacgaacgaagagcgattgaggaaaaggcggcggcggccggcatgagcctgtcggcctacctgctggccgtcggccagggctacaaaatcacgggcgtcgtggactatgagcacgtccgcgagggcgtcccggaaaacgattccgaagcccaacctttcatagaaggcggcggtggaatcgaaatctcgtgatggcaggttgggcgtcgcttggtcggtcatttcgaaaaaggttaggaatacggttagccatttgcctgcttttatatagttcatatgggattcacctttatgttgataagaaataaaagaaaatgccaataggatatcggcattttcttttgcgtttttatttgttaactgttaattgtccttgttcaaggatgctgtctttgacaacagatgttttcttgcctttgatgttcagcaggaagctcggcgcaaacgttgattgtttgtctgcgtagaatcctctgtttgtcatatagcttgtaatcacgacattgtttcctttcgcttgaggtacagcgaagtgtgagtaagtaaaggttacatcgttaggcggatcaagatccatttttaacacaaggccagttttgttcagcggcttgtatgggccagttaaagaattagaaacataaccaagcatgtaaatatcgttagacgtaatgccgtcaatcgtcatttttgatccgcgggagtcagtgaacaggtaccatttgccgttcattttaaagacgttcgcgcgttcaatttcatctgttactgtgttagatgcaatcagcggtttcatcacttttttcagtgtgtaatcatcgtttagctcaatcataccgagagcgccgtttgctaactcagccgtgcgttttttatcgctttgcagaagtttttgactttcttgacggaagaatgatgtgcttttgccatagtatgctttgttaaataaagattcttcgccttggtagccatcttcagttccagtgtttgcttcaaatactaagtatttgtggcctttatcttctacgtagtgaggatctctcagcgtatggttgtcgcctgagctgtagttgccttcatcgatgaactgctgtacattttgatacgtttttccgtcaccgtcaaagattgatttataatcctctacaccgttgatgttcaaagagctgtctgatgctgatacgttaacttgtgcagttgtcagtgtttgtttgccgtaatgtttaccggagaaatcagtgtagaataaacggatttttccgtcagatgtaaatgtggctgaacctgaccattcttgtgtttggtcttttaggatagaatcatttgcatcgaatttgtcgctgtctttaaagacgcggccagcgtttttccagctgtcaatagaagtttcgccgactttttgatagaacatgtaaatcgatgtgtcatccgcatttttaggatctccggctaatgcaaagacgatgtggtagccgtgatagtttgcgacagtgccgtcagcgttttgtaatggccagctgtcccaaacgtccaggccttttgcagaagagatatttttaattgtggacgaatcaaattcagaaacttgatatttttcatttttttgctgttcagggatttgcagcatatcatggcgtgtaatatgggaaatgccgtatgtttccttatatggcttttggttcgtttctttcgcaaacgcttgagttgcgcctcctgccagcagtgcggtagtaaaggttaatactgttgcttgttttgcaaactttttgatgttcatcgttcatgtctccttttttatgtactgtgttagcggtctgcttcttccagccctcctgtttgaagatggcaagttagttacgcacaataaaaaaagacctaaaatatgtaaggggtgacgccaaagtatacactttgccctttacacattttaggtcttgcctgctttatcagtaacaaacccgcgcgatttacttttcgacctcattctattagactctcgtttggattgcaactggtctattttcctcttttgtttgatagaaaatcataaaaggatttgcagactacgggcctaaagaactaaaaaatctatctgtttcttttcattctctgtattttttatagtttctgttgcatgggcataaagttgcctttttaatcacaattcagaaaatatcataatatctcatttcactaaataatagtgaacggcaggtatatgtgatgggttaaaaaggatcaccccagagtcccgctcagaagaactcgtcaagaaggcgatagaaggcgatgcgctgcgaatcgggagcggcgataccgtaaagcacgaggaagcggtcagcccattcgccgccaagctcttcagcaatatcacgggtagccaacgctatgtcctgatagcggtccgccacacccagccggccacagtcgatgaatccagaaaagcggccattttccaccatgatattcggcaagcaggcatcgccatgggtcacgacgagatcctcgccgtcgggcatccgcgccttgagcctggcgaacagttcggctggcgcgagcccctgatgctcttcgtccagatcatcctgatcgacaagaccggcttccatccgagtacgtgctcgctcgatgcgatgtttcgcttggtggtcgaatgggcaggtagccggatcaagcgtatgcagccgccgcattgcatcagccatgatggatactttctcggcaggagcaaggtgagatgacaggagatcctgccccggcacttcgcccaatagcagccagtcccttcccgcttcagtgacaacgtcgagacagctgcgcaaggaacgcccgtcgtggccagccacgatagccgcgctgcctcgtcttggagttcattcagggcaccggacaggtcggtcttgacaaaaagaaccgggcgcccctgcgctgacagccggaacacggcggcatcagagcagccgattgtctgttgtgcccagtcatagccgaatagcctctccacccaagcggccggagaacctgcgtgcaatccatcttgttcaatcatgcgaaacgatcctcatcctgtctcttgatcagatcttgatcccctgcgccatcagatccttggcggcaagaaagccatccagtttactttgcagggcttcccaaccttaccagagggcgccccagctggcaattccg